European Patent Application EP 4 249 501 A2, published September 27, 2023. Title: METHODS OF ALTERING GENE EXPRESSION BY PERTURBING TRANSCRIPTION FACTOR MULTIMERS THAT STRUCTURE REGULATORY LOOPS. Applicant: WHITEHEAD INSTITUTE FOR BIOMEDICAL RESEARCH. Application EP, filed January 9, 2018. The sequence listing filed with the application follows.

SEQUENCE LISTING (45 sequences)

SEQ ID NO: 1 - RNA, 20 nt, synthetic construct
  misc_feature 1..20: note = Guide RNA
  source 1..20: mol_type = other RNA
actgtcaatgtaggcccata

SEQ ID NO: 2 - DNA, 40 bp, Mus musculus
  source 1..40: mol_type = unassigned DNA
gcgtcggccatgacagttacatccgggtatgatgcctagc

SEQ ID NO: 3 - DNA, 35 bp, Mus musculus
  source 1..35: mol_type = unassigned DNA
gcgtcggcctgtgacatccgggtatgatgcctagc

SEQ ID NO: 4 - DNA, 25 bp, Mus musculus
  source 1..25: mol_type = unassigned DNA
cgggtgctggtgccgccatcttgga

SEQ ID NO: 5 - DNA, 12 bp, Mus musculus
  source 1..12: mol_type = unassigned DNA
cgggtgcttgga

SEQ ID NO: 6 - DNA, 22 bp, Mus musculus
  source 1..22: mol_type = unassigned DNA
actgtgcctccatttgttttca

SEQ ID NO: 7 - DNA, 12 bp, Mus musculus
  source 1..12: mol_type = unassigned DNA
actgtgttttca

SEQ ID NO: 8 - DNA, 25 bp, synthetic construct
  misc_feature 1..25: note = primer
  source 1..25: mol_type = other DNA
caccgactcccgccatccaagatgg

SEQ ID NO: 9 - DNA, 25 bp, synthetic construct
  misc_feature 1..25: note = primer
  source 1..25: mol_type = other DNA
aaacccatcttggatggcgggagtc

SEQ ID NO: 10 - DNA, 25 bp, synthetic construct
  misc_feature 1..25: note = primer
  source 1..25: mol_type = other DNA
caccgagctacttgaaaacaaatgg

SEQ ID NO: 11 - DNA, 25 bp, synthetic construct
  misc_feature 1..25: note = primer
  source 1..25: mol_type = other DNA
aaacccatttgttttcaagtagctc

SEQ ID NO: 12 - DNA, 24 bp, synthetic construct
  misc_feature 1..24: note = primer
  source 1..24: mol_type = other DNA
caccgtcttctctcttcttttcac

SEQ ID NO: 13 - DNA, 24 bp, synthetic construct
  misc_feature 1..24: note = primer
  source 1..24: mol_type = other DNA
aaacgtgaaaagaagagagaagac

SEQ ID NO: 14 - DNA, 20 bp, synthetic construct
  misc_feature 1..20: note = primer
  source 1..20: mol_type = other DNA
ctgtgcagtgattgggtcct

SEQ ID NO: 15 - DNA, 20 bp, synthetic construct
  misc_feature 1..20: note = primer
  source 1..20: mol_type = other DNA
ttgccgctctgcacttaagt

SEQ ID NO: 16 - DNA, 22 bp, synthetic construct
  misc_feature 1..22: note = primer
  source 1..22: mol_type = other DNA
gcttcctcacattgaaacagaa

SEQ ID NO: 17 - DNA, 22 bp, synthetic construct
  misc_feature 1..22: note = primer
  source 1..22: mol_type = other DNA
gggaagctctgagagtccttat

SEQ ID NO: 18 - DNA, 17 bp, synthetic construct
  misc_feature 1..17: note = primer
  source 1..17: mol_type = other DNA
cgccaccaggatgacag

SEQ ID NO: 19 - DNA, 19 bp, synthetic construct
  misc_feature 1..19: note = primer
  source 1..19: mol_type = other DNA
gaatgtgaccgcaaccaac

SEQ ID NO: 20 - DNA, 20 bp, synthetic construct
  misc_feature 1..20: note = primer
  source 1..20: mol_type = other DNA
cattttacctgcccccagta

SEQ ID NO: 21 - DNA, 20 bp, synthetic construct
  misc_feature 1..20: note = primer
  source 1..20: mol_type = other DNA
cagccttaaacagcctggaa

SEQ ID NO: 22 - DNA, 20 bp, synthetic construct
  misc_feature 1..20: note = primer
  source 1..20: mol_type = other DNA
tttcaaagccaccaaggtct

SEQ ID NO: 23 - DNA, 20 bp, synthetic construct
  misc_feature 1..20: note = primer
  source 1..20: mol_type = other DNA
caagtagctcggggtctcag

SEQ ID NO: 24 - DNA, 19 bp, synthetic construct
  misc_feature 1..19: note = Bridge linker
  misc_feature 1: note = 5' phosphorylation
  misc_feature 10: note = biotinylation
  source 1..19: mol_type = other DNA
cgcgatatcttatctgact

SEQ ID NO: 25 - DNA, 19 bp, synthetic construct
  misc_feature 1..19: note = bridge linker
  misc_feature 1: note = 5' phosphorylation
  source 1..19: mol_type = other DNA
gtcagataagatatcgcgt

SEQ ID NO: 26 - DNA, 22 bp, synthetic construct
  misc_feature 1..22: note = primer
  source 1..22: mol_type = other DNA
gtctggatcctcgtcttgagcc

SEQ ID NO: 27 - DNA, 22 bp, synthetic construct
  misc_feature 1..22: note = primer
  source 1..22: mol_type = other DNA
ccaaggatccgtaagctaggct

SEQ ID NO: 28 - DNA, 199 bp, synthetic construct
  misc_feature 1..199: note = competitor DNA
  source 1..199: mol_type = other DNA
gagcaacaacaacaacgaaccggttcgacctccccggccatctttcgacctccccggccatctttcgacctccccggccatctttcgacctccccggccatctttcgacctccccggccatctttcgacctccccggccatctttcgacctccccggccatctttcgacctcccgtcgacagaggcagcaaaagccaga

SEQ ID NO: 29 - DNA, 20 bp, synthetic construct
  misc_feature 1..20: note = primer
  source 1..20: mol_type = other DNA
caagggcaagtaacccgatc

SEQ ID NO: 30 - DNA, 20 bp, synthetic construct
  misc_feature 1..20: note = primer
  source 1..20: mol_type = other DNA
aatagatacatcccccacct

SEQ ID NO: 31 - DNA, 20 bp, synthetic construct
  misc_feature 1..20: note = primer
  source 1..20: mol_type = other DNA
caagggcaagtaacccgatc

SEQ ID NO: 32 - DNA, 20 bp, synthetic construct
  misc_feature 1..20: note = primer
  source 1..20: mol_type = other DNA
aatagatacatcccccacct

SEQ ID NO: 33 - DNA, 30 bp, synthetic construct
  misc_feature 1..30: note = primer
  source 1..30: mol_type = other DNA
tcgctccccggccatcttggcggctggtgt

SEQ ID NO: 34 - DNA, 30 bp, synthetic construct
  misc_feature 1..30: note = primer
  source 1..30: mol_type = other DNA
acaccagccgccaagatggccggggagcga

SEQ ID NO: 35 - DNA, 25 bp, synthetic construct
  misc_feature 1..25: note = primer
  source 1..25: mol_type = other DNA
caccgaagtagctcggggtctcaga

SEQ ID NO: 36 - DNA, 25 bp, synthetic construct
  misc_feature 1..25: note = primer
  source 1..25: mol_type = other DNA
aaactctgagaccccgagctacttc

SEQ ID NO: 37 - DNA, 24 bp, synthetic construct
  misc_feature 1..24: note = primer
  source 1..24: mol_type = other DNA
caccggtgctcagtaaatgtaaac

SEQ ID NO: 38 - DNA, 24 bp, synthetic construct
  misc_feature 1..24: note = primer
  source 1..24: mol_type = other DNA
aaacgtttacatttactgagcacc

SEQ ID NO: 39 - DNA, 23 bp, Mus musculus
  source 1..23: mol_type = unassigned DNA
actcccgccatccaagatggcgg

SEQ ID NO: 40 - DNA, 24 bp, Mus musculus
  source 1..24: mol_type = unassigned DNA
gagctacttgaaaacaaatggagg

SEQ ID NO: 41 - DNA, 23 bp, Mus musculus
  source 1..23: mol_type = unassigned DNA
gtcttctctcttcttttcactgg

SEQ ID NO: 42 - DNA, 20 bp, synthetic construct
  misc_feature 1..20: note = linker sequence
  source 1..20: mol_type = other DNA
acgcgatatcttatctgact

SEQ ID NO: 43 - DNA, 20 bp, synthetic construct
  misc_feature 1..20: note = linker sequence
  source 1..20: mol_type = other DNA
agtcagataagatatcgcgt

SEQ ID NO: 44 - DNA, 11 bp, synthetic construct
  misc_feature 1..11: note = YY1 binding motif
  misc_feature 9: note = n is a, c, t, or g
  source 1..11: mol_type = other DNA
ggcgccatntt

SEQ ID NO: 45 - DNA, 12 bp, synthetic construct
  misc_feature 1..12: note = YY1 binding motif
  source 1..12: mol_type = other DNA
gccgccattttg